European Patent Application EP 4 215 212 A1, published July 26, 2023. Title: Composition for treating or preventing diseases, disorders or symptoms associated with endoplasmic reticulum stress or all-trans-retinal, or for protecting retinal thickness or inhibiting atrophy or atrophy progression of retinal thickness. Applicant: RESTORE VISION INC. The sequence listing filed with the application follows.

SEQUENCE LISTING (25 sequences)

SEQ ID NO: 1 - DNA, 1078 bp, artificial sequence
  An example of nucleic acid sequence consisting of chimera rhodopsin (GR/BvRh) and ER export signal
ctggatccgatatcaagcttgccaccatgctgatgaccgtgttcagcagcgcccctgagctggccctgctgggctctacatttgcccaggtggaccccagcaacctgagcgtgtccgacagcctgacctacggccagttcaacctggtgtacaacgccttcagcttcgccattgccgccatgttcgccagcgccctgttcttcttcagtgcacaagccctcgtgggccagcggtacagactggctctgctggtgtctgccatcgtggtgtctatcgccggctaccactacttccggatcttcaacagctgggacgccgcctacgtgctggaaaacggcgtgtactccctgaccagcgagaagttcaacgacgcctacagatacgtggactggctgctgaccgtgcccctgctgctggtgcaaacagtggccgtgatcgagcgctacgtggtcgtgtgcaagcccatgagcaacttcagattcggcgagaaccaccccctgctgatcaagctgacagtggccagcgtgctgatgatcgccacaggctaccctggcgagatcagcgacgacatcaccacccggatcatctggggaaccgtgtccaccatccccttcgcctacatcctgtacgtgctgtgggtggaactgagcttcaccgtgaaagaggccgctgctcagcagcaggaaagcgccacaacccaggtgcagaccctcgtgcggaacatgagatggttgctgctgctgtcctggggcgtgtaccctatcgcctacctgctgcctatgctgggcgtgtccggaacatctgccgctgtgggagtgcaagtgggctacacaatcgccgatgtgctggccaagcccgtgttcggcctgctggtgttcgctatcgccctcgtgaaaacaaaggccgaccaggaaagcagcgagccccacgccgctattggagccgccgctaacaagtctggcggcagcctgatcagcggatccgccagcgccagcaacggcgccagcgaattcttctgctacgagaatgaagtgtaatctagcgagctcctcgagtaatcaacctctggattacaaaa

SEQ ID NO: 2 - protein, 336 aa, artificial sequence
  An example of amino acid sequence consisting of chimera rhodopsin (GR/BvRh) and ER export signal
MLMTVFSSAPELALLGSTFAQVDPSNLSVSDSLTYGQFNLVYNAFSFAIAAMFASALFFFSAQALVGQRYRLALLVSAIVVSIAGYHYFRIFNSWDAAYVLENGVYSLTSEKFNDAYRYVDWLLTVPLLLVQTVAVIERYVVVCKPMSNFRFGENHPLLIKLTVASVLMIATGYPGEISDDITTRIIWGTVSTIPFAYILYVLWVELSFTVKEAAAQQQESATTQVQTLVRNMRWLLLLSWGVYPIAYLLPMLGVSGTSAAVGVQVGYTIADVLAKPVFGLLVFAIALVKTKADQESSEPHAAIGAAANKSGGSLISGSASASNGASEFFCYENEV

SEQ ID NO: 3 - DNA, 1102 bp, artificial sequence
  An example of nucleic acid sequence consisting of chimera rhodopsin (GR/BvRh), ER export signal and FLAG tag
ctggatccgatatcaagcttgccaccatgctgatgaccgtgttcagcagcgcccctgagctggccctgctgggctctacatttgcccaggtggaccccagcaacctgagcgtgtccgacagcctgacctacggccagttcaacctggtgtacaacgccttcagcttcgccattgccgccatgttcgccagcgccctgttcttcttcagtgcacaagccctcgtgggccagcggtacagactggctctgctggtgtctgccatcgtggtgtctatcgccggctaccactacttccggatcttcaacagctgggacgccgcctacgtgctggaaaacggcgtgtactccctgaccagcgagaagttcaacgacgcctacagatacgtggactggctgctgaccgtgcccctgctgctggtgcaaacagtggccgtgatcgagcgctacgtggtcgtgtgcaagcccatgagcaacttcagattcggcgagaaccaccccctgctgatcaagctgacagtggccagcgtgctgatgatcgccacaggctaccctggcgagatcagcgacgacatcaccacccggatcatctggggaaccgtgtccaccatccccttcgcctacatcctgtacgtgctgtgggtggaactgagcttcaccgtgaaagaggccgctgctcagcagcaggaaagcgccacaacccaggtgcagaccctcgtgcggaacatgagatggttgctgctgctgtcctggggcgtgtaccctatcgcctacctgctgcctatgctgggcgtgtccggaacatctgccgctgtgggagtgcaagtgggctacacaatcgccgatgtgctggccaagcccgtgttcggcctgctggtgttcgctatcgccctcgtgaaaacaaaggccgaccaggaaagcagcgagccccacgccgctattggagccgccgctaacaagtctggcggcagcctgatcagcggatccgccagcgccagcaacggcgccagcgactacaaagacgatgacgacaaggaattcttctgctacgagaatgaagtgtaatctagcgagctcctcgagtaatcaacctctggattacaaaa

SEQ ID NO: 4 - protein, 344 aa, artificial sequence
  An example of amino acid sequence consisting of chimera rhodopsin (GR/BvRh), ER export signal and FLAG tag
MLMTVFSSAPELALLGSTFAQVDPSNLSVSDSLTYGQFNLVYNAFSFAIAAMFASALFFFSAQALVGQRYRLALLVSAIVVSIAGYHYFRIFNSWDAAYVLENGVYSLTSEKFNDAYRYVDWLLTVPLLLVQTVAVIERYVVVCKPMSNFRFGENHPLLIKLTVASVLMIATGYPGEISDDITTRIIWGTVSTIPFAYILYVLWVELSFTVKEAAAQQQESATTQVQTLVRNMRWLLLLSWGVYPIAYLLPMLGVSGTSAAVGVQVGYTIADVLAKPVFGLLVFAIALVKTKADQESSEPHAAIGAAANKSGGSLISGSASASNGASDYKDDDDKEFFCYENEV

SEQ ID NO: 5 - protein, 317 aa, artificial sequence
  An example of amino acid sequence encoding chimera rhodopsin (GR/BvRh)
MLMTVFSSAPELALLGSTFAQVDPSNLSVSDSLTYGQFNLVYNAFSFAIAAMFASALFFFSAQALVGQRYRLALLVSAIVVSIAGYHYFRIFNSWDAAYVLENGVYSLTSEKFNDAYRYVDWLLTVPLLLVQTVAVIERYVVVCKPMSNFRFGENHPLLIKLTVASVLMIATGYPGEISDDITTRIIWGTVSTIPFAYILYVLWVELSFTVKEAAAQQQESATTQVQTLVRNMRWLLLLSWGVYPIAYLLPMLGVSGTSAAVGVQVGYTIADVLAKPVFGLLVFAIALVKTKADQESSEPHAAIGAAANKSGGSLIS

SEQ ID NO: 6 - DNA, 939 bp, artificial sequence
  An example of nucleic acid sequence encoding chimera rhodopsin (GtACR2/BvRh)
aagcttatggccagccaggtggtgtacggcgagtgggcctctacccacaccgagtgctacaacatgagccggatcgacagcaccttcgtgtccctgctgcagctcgtgtgggccgtggtgtctggctgtcagaccatcttcatgatcagcagagcccccaaggtgccctgggagagcgtgtacctgcccttcgtggaatccatcacctacgccctggccagcaccggcaatggcacactgcagatgcgggacggccggttcttcccttggtcacggatggcctcttggctgtgcacctgtcccatcatgctgggccagatcagcaacatgatcgagagatacgtggtcgtgtgcaagcccatgagcaacttcagattcggcgagaaccacatccccctgaaccctattgcccaggccgccagcatcatccgggtcgtgatgggcatcaccgccaccattagccctgccgagtatatgaagtggctgttcttcttcttcggcgccacctgtctggtgttcgagtacagcgtggtgttcaccatcttccaagtgggcctgttcaccgtgaaagaggccgctgcccagcagcaggaaagcgccacaacacaggcccagaaagtggtcgtgcggatcaagatgctgcggctgatcttctttatcgcctggaccatgttccccatcgtgtggctgatctcccccaccggcgtgtgcgtgatccacgagaatgtgtccgccatcctgtacctgctggccgacggcctgtgcaagaacacctacggcgtgatcctgtggtccaccgcctggggagtgctggaaggcaaatgggaccctgcctgtctgcccggccaggaaaaacctgaggccgacgatcccttcggcctgaaccacgagaagaacgcccctcccaacgacgaagtgaacatcagaatgttcggcagg

SEQ ID NO: 7 - DNA, 1374 bp, artificial sequence
  An example of nucleic acid sequence encoding chimera rhodopsin (GtACR2/BvRh)
atggcaagccaagtcgtttatggagaatgggcgagtacgcatacagaatgttacaacatgtcaaggatcgacagcacctttgtctcattgctgcagctggtctgggctgttgtcagcggatgccagacgatctttatgatctctcgagccccgaaggtgccatgggaatctgtttaccttcccttcgttgaaagcatcacctatgccctcgcttctactggaaacggcacgttgcagatgagggacgggcgcttctttccttggtcgcgcatggcatcctggttgtgcacttgccctatcatgctcgggcagatcagcaacatgatcgagcggtacgtagtggtgtgcaagcccatgagcaacttccgcttcggggagaaccacatcccgttgaatcccatcgcgcaagcagcctccatcatccgagtggtgatgggaatcacggcgactatctctcccgccgagtacatgaagtggctctttttcttcttcggggccacgtgcctggtctttgagtactcagttgtcttcaccatctttcaagtcgggctgttcaccgtcaaggaggctgcagcccagcagcaggagtcggccaccactcaggctcagaaggtggtggtgagaatcaagatgctcagactcatcttcttcatcgcatggaccatgttccccatcgtatggctgatatcccccactggcgtctgcgtcattcatgagaacgtgagcgctatcctgtacctcctcgccgacgggctctgcaagaacacctacggagtgatcctgtggagcacggcatggggcgtgttggaagggaagtgggaccctgcatgccttccaggacaggagaagccggaggccgacgatccgtttgggctgaaccatgagaagaatgctccccccaacgatgaagtcaacatccggatgttcggagtcatcggctcggtgaggaagtcaaagaggaggcagaagtgggagctggcgccggcgcatctagaggacaggatcaggttgagcgacgaggagtcggatgactcgaggccgaagaggaagaagaaaggagacgcgcgggactacaggaggaagcatcgaggaggcgccgacgacgacgatcatcacagcagcgaatcggagagtgagaagaagaacaagggaaagaagaagaagtcgggcaagggaaagaagaaggacgactcgggctccgaggacgatcttgaggtcggcaacgggaaggcgaagaacggagacaagcaggagttcaacgacatcaacaagatcctacgagccatgaagagaaacgccgggacgctgagcgaaaagtctcattccgatgactccgagggaaagcgtgagagcgcggatcattccatgtgctga

SEQ ID NO: 8 - protein, 311 aa, Artificial Sequence
  An example of amino acid sequence encoding chimera rhodopsin (GtACR2/BvRh)
MASQVVYGEWASTHTECYNMSRIDSTFVSLLQLVWAVVSGCQTIFMISRAPKVPWESVYLPFVESITYALASTGNGTLQMRDGRFFPWSRMASWLCTCPIMLGQISNMIERYVVVCKPMSNFRFGENHIPLNPIAQAASIIRVVMGITATISPAEYMKWLFFFFGATCLVFEYSVVFTIFQVGLFTVKEAAAQQQESATTQAQKVVVRIKMLRLIFFIAWTMFPIVWLISPTGVCVIHENVSAILYLLADGLCKNTYGVILWSTAWGVLEGKWDPACLPGQEKPEADDPFGLNHEKNAPPNDEVNIRMFGR

SEQ ID NO: 9 - DNA, 1047 bp, Homo sapiens
atgaatggcacagaaggccctaacttctacgtgcccttctccaatgcgacgggtgtggtacgcagccccttcgagtacccacagtactacctggctgagccatggcagttctccatgctggccgcctacatgtttctgctgatcgtgctgggcttccccatcaacttcctcacgctctacgtcaccgtccagcacaagaagctgcgcacgcctctcaactacatcctgctcaacctagccgtggctgacctcttcatggtcctaggtggcttcaccagcaccctctacacctctctgcatggatacttcgtcttcgggcccacaggatgcaatttggagggcttctttgccaccctgggcggtgaaattgccctgtggtccttggtggtcctggccatcgagcggtacgtggtggtgtgtaagcccatgagcaacttccgcttcggggagaaccatgccatcatgggcgttgccttcacctgggtcatggcgctggcctgcgccgcacccccactcgccggctggtccaggtacatccccgagggcctgcagtgctcgtgtggaatcgactactacacgctcaagccggaggtcaacaacgagtcttttgtcatctacatgttcgtggtccacttcaccatccccatgattatcatctttttctgctatgggcagctcgtcttcaccgtcaaggaggccgctgcccagcagcaggagtcagccaccacacagaaggcagagaaggaggtcacccgcatggtcatcatcatggtcatcgctttcctgatctgctgggtgccctacgccagcgtggcattctacatcttcacccaccagggctccaacttcggtcccatcttcatgaccatcccagcgttctttgccaagagcgccgccatctacaaccctgtcatctatatcatgatgaacaagcagttccggaactgcatgctcaccaccatctgctgcggcaagaacccactgggtgacgatgaggcctctgctaccgtgtccaagacggagacgagccaggtggccccggcctaa

SEQ ID NO: 10 - protein, 348 aa, Homo sapiens [sequence omitted]

SEQ ID NO: 11 - DNA, 1047 bp, Bos taurus
atgaacgggaccgagggcccaaacttctacgtgcctttctccaacaagacgggcgtggtgcgcagccccttcgaggccccgcagtactacctggcggagccatggcagttctccatgctggccgcctacatgttcctgctgatcatgcttggcttccccatcaacttcctcacgctgtacgtcacagtccagcacaagaagctgcgcacacccctcaactacatcctgctcaacctggccgtggccgacctcttcatggtcttcgggggcttcaccaccaccctctacacctctctgcacggatacttcgtctttgggcccacgggctgcaacctggagggcttctttgccaccctgggcggtgaaattgcactgtggtccttggtggtcctggccatcgagcggtacgtggtggtgtgcaagcccatgagcaacttccgcttcggggagaaccacgccatcatgggcgtcgccttcacctgggtcatggctctggcctgtgccgcgccccccctcgtcggctggtccaggtacatcccggagggcatgcagtgctcgtgcgggattgactactacacgccccacgaggagaccaacaatgagtcgttcgtcatctacatgttcgtggtccacttcatcatccccctgattgtcatattcttctgctacgggcagctggtgttcaccgtcaaggaggcggctgcccagcagcaggagtcggccaccactcagaaggccgagaaggaggtcacccgcatggtgatcatcatggtcatcgctttcctaatctgctggctgccctacgctggggtggcgttctacatcttcacccatcagggctctgactttggccccatcttcatgaccatcccggctttctttgccaagacttctgccgtctacaaccccgtcatctacatcatgatgaacaagcagttccggaactgcatggtcaccactctctgctgtggcaagaacccgctgggtgacgacgaggcctccaccaccgtctccaagacagagaccagccaggtggcgcctgcctaa

SEQ ID NO: 12 - protein, 348 aa, Bos taurus
MNGTEGPNFYVPFSNKTGVVRSPFEAPQYYLAEPWQFSMLAAYMFLLIMLGFPINFLTLYVTVQHKKLRTPLNYILLNLAVADLFMVFGGFTTTLYTSLHGYFVFGPTGCNLEGFFATLGGEIALWSLVVLAIERYVVVCKPMSNFRFGENHAIMGVAFTWVMALACAAPPLVGWSRYIPEGMQCSCGIDYYTPHEETNNESFVIYMFVVHFIIPLIVIFFCYGQLVFTVKEAAAQQQESATTQKAEKEVTRMVIIMVIAFLICWLPYAGVAFYIFTHQGSDFGPIFMTIPAFFAKTSAVYNPVIYIMMNKQFRNCMVTTLCCGKNPLGDDEASTTVSKTETSQVAPA

SEQ ID NO: 13 - DNA, 897 bp, Gloeobacter violaceus
atgttgatgaccgtattttcttctgcacctgaacttgcccttctcggatcaacctttgcccaggtcgatccttcaaacttatcggtctcagattcgctgacctatggtcagttcaatctggtttacaacgctttctcgtttgccatcgcggcaatgttcgcatctgccctcttcttcttcagcgctcaggcactcgtcggtcaacgataccggttggccttgcttgtttcagcaattgttgtgagtatcgctgggtaccactactttcggatcttcaatagttgggatgctgcctacgttctggagaatggcgtgtattccctgactagcgaaaaattcaacgacgcctaccgctatgtggattggctgttgaccgtgcctctgttgctggtggagacagtggcagtgctgacgttgcctgcaaaggaggcaagacccttgctgatcaaactgacggtggcttcagttctgatgattgccacgggctaccccggcgagatttctgacgacattacgactcgcatcatctggggtacggtcagcacgattcccttcgcctacatcctctatgtgttgtgggtcgaactgtccaggtcccttgtccgccagcccgctgctgtacaaaccctggtccgcaacatgcggtggctgctgttgctctcctggggtgtttacccgatcgcataccttctacccatgcttggagtatccggtacgtccgcggctgtcggcgttcaggttggctatacgatcgcagacgtgctggcgaagcctgtatttggtcttctagtcttcgcgattgcactcgtgaaaacaaaagcagatcaagaaagcagtgaaccacatgccgcaataggtgctgctgcaaataaatcgggaggcagtcttatctcctag

SEQ ID NO: 14 - protein, 298 aa, Gloeobacter violaceus
MLMTVFSSAPELALLGSTFAQVDPSNLSVSDSLTYGQFNLVYNAFSFAIAAMFASALFFFSAQALVGQRYRLALLVSAIVVSIAGYHYFRIFNSWDAAYVLENGVYSLTSEKFNDAYRYVDWLLTVPLLLVETVAVLTLPAKEARPLLIKLTVASVLMIATGYPGEISDDITTRIIWGTVSTIPFAYILYVLWVELSRSLVRQPAAVQTLVRNMRWLLLLSWGVYPIAYLLPMLGVSGTSAAVGVQVGYTIADVLAKPVFGLLVFAIALVKTKADQESSEPHAAIGAAANKSGGSLIS

SEQ ID NO: 15 - DNA, 1317 bp, Guillardia theta
atggcaagccaagtcgtttatggagaatgggcgagtacgcatacagaatgttacaacatgtcaaggatcgacagcacctttgtctcattgctgcagctggtctgggctgttgtcagcggatgccagacgatctttatgatctctcgagccccgaaggtgccatgggaatctgtttaccttcccttcgttgaaagcatcacctatgccctcgcttctactggaaacggcacgttgcagatgagggacgggcgcttctttccttggtcgcgcatggcatcctggttgtgcacttgccctatcatgctcgggcagatcagcaacatggcgctggtgaagtacaagagcatcccgttgaatcccatcgcgcaagcagcctccatcatccgagtggtgatgggaatcacggcgactatctctcccgccgagtacatgaagtggctctttttcttcttcggggccacgtgcctggtctttgagtactcagttgtcttcaccatctttcaagtcgggctgtacgggtttgagagcgtggggactccgctggctcagaaggtggtggtgagaatcaagatgctcagactcatcttcttcatcgcatggaccatgttccccatcgtatggctgatatcccccactggcgtctgcgtcattcatgagaacgtgagcgctatcctgtacctcctcgccgacgggctctgcaagaacacctacggagtgatcctgtggagcacggcatggggcgtgttggaagggaagtgggaccctgcatgccttccaggacaggagaagccggaggccgacgatccgtttgggctgaaccatgagaagaatgctccccccaacgatgaagtcaacatccggatgttcggacgcgtcatcggctcggtgaggaagtcaaagaggaggcagaagtgggagctggcgccggcgcatctagaggacaggatcaggttgagcgacgaggagtcggatgactcgaggccgaagaggaagaagaaaggagacgcgcgggactacaggaggaagcatcgaggaggcgccgacgacgacgatcatcacagcagcgaatcggagagtgagaagaagaacaagggaaagaagaagaagtcgggcaagggaaagaagaaggacgactcgggctccgaggacgatcttgaggtcggcaacgggaaggcgaagaacggagacaagcaggagttcaacgacatcaacaagatcctacgagccatgaagagaaacgccgggacgctgagcgaaaagtctcattccgatgactccgagggaaagcgtgagagcgcggatcattccatgtgctga

SEQ ID NO: 16 - protein, 438 aa, Guillardia theta
MASQVVYGEWASTHTECYNMSRIDSTFVSLLQLVWAVVSGCQTIFMISRAPKVPWESVYLPFVESITYALASTGNGTLQMRDGRFFPWSRMASWLCTCPIMLGQISNMALVKYKSIPLNPIAQAASIIRVVMGITATISPAEYMKWLFFFFGATCLVFEYSVVFTIFQVGLYGFESVGTPLAQKVVVRIKMLRLIFFIAWTMFPIVWLISPTGVCVIHENVSAILYLLADGLCKNTYGVILWSTAWGVLEGKWDPACLPGQEKPEADDPFGLNHEKNAPPNDEVNIRMFGRVIGSVRKSKRRQKWELAPAHLEDRIRLSDEESDDSRPKRKKKGDARDYRRKHRGGADDDDHHSSESESEKKNKGKKKKSGKGKKKDDSGSEDDLEVGNGKAKNGDKQEFNDINKILRAMKRNAGTLSEKSHSDDSEGKRESADHSMC

SEQ ID NO: 17 - DNA, 34 bp, artificial sequence
  Artificial Nucleic Acid
atcgagcgctacgtggtcgtgtgcaagcccatga

SEQ ID NO: 18 - DNA, 33 bp, artificial sequence
  Artificial Nucleic Acid
atcgagcggtacgtagtggtgtgcaagcccatg

SEQ ID NO: 19 - protein, 11 aa, artificial sequence
  Artificial Peptide
IERYVVVCKPM

SEQ ID NO: 20 - DNA, 51 bp, artificial sequence
  Artificial Nucleic Acid
ttcaccgtgaaagaggccgctgctcagcagcaggaaagcgccacaacccag

SEQ ID NO: 21 - DNA, 51 bp, artificial sequence
  Artificial Nucleic Acid
ttcaccgtcaaggaggctgcagcccagcagcaggagtcggccaccactcag

SEQ ID NO: 22 - protein, 16 aa, artificial sequence
  Artificial Peptide
FTVKEAAAQQQESATT

SEQ ID NO: 23 - DNA, 1036 bp, artificial sequence
  Artificial Nucleic Acid
ggagacccaagctggctagcgtttaaacttaagcttgccaccatgttgatgaccgtattttcttctgcacctgaacttgcccttctcggatcaacctttgcccaggtcgatccttcaaacttatcggtctcagattcgctgacctatggtcagttcaatctggtttacaacgctttctcgtttgccatcgcggcaatgttcgcatctgccctcttcttcttcagcgctcaggcactcgtcggtcaacgataccggttggccttgcttgtttcagcaattgttgtgagtatcgctgggtaccactactttcggatcttcaatagttgggatgctgcctacgttctggagaatggcgtgtattccctgactagcgaaaaattcaacgacgcctaccgctatgtggattggctgttgaccgtgcctctgttgctggtgcaaacagtggcagtgatcgagcggtacgtagtggtgtgcaagcccatgagcaacttccgcttcggggagaaccaccccttgctgatcaaactgacggtggcttcagttctgatgattgccacgggctaccccggcgagatttctgacgacattacgactcgcatcatctggggtacggtcagcacgattcccttcgcctacatcctctatgtgttgtgggtcgaactgtccttcaccgtcaaggaggctgcagcccagcagcaggagtcggccaccactcaggtacaaaccctggtccgcaacatgcggtggctgctgttgctctcctggggtgtttacccgatcgcataccttctacccatgcttggagtatccggtacgtccgcggctgtcggcgttcaggttggctatacgatcgcagacgtgctggcgaagcctgtatttggtcttctagtcttcgcgattgcactcgtgaaaacaaaagcagatcaagaaagcagtgaaccacatgccgcaataggtgctgctgcaaataaatcgggaggcagtcttatctcctgatctagagggcccgtttaaacccgctgatcagcctcgactg

SEQ ID NO: 24 - DNA, 60 bp, artificial sequence
  Artificial Nucleic Acid
atcgagcggtacgtagtggtgtgcaagcccatgagcaacttccgcttcggggagaaccac

SEQ ID NO: 25 - protein, 20 aa, artificial sequence
  Artificial Peptide
IERYVVVCKPMSNFRFGENH